European Patent Specification EP 4 029 951 B1, published February 5, 2025. Title: METHOD AND PRIMERS FOR DETECTING DHA CANOLA NS-50027-4. Applicant: Nuseed Nutritional Australia Pty Ltd. The sequence listing filed with the application follows.

SEQUENCE LISTING (11 sequences)

SEQ ID NO: 1 - DNA, 21 bp, Artificial Sequence
  Forward primer for A05-216 assay (A05-216F)
agattgtcgtttcccgccttc

SEQ ID NO: 2 - DNA, 19 bp, Artificial Sequence
  Reverse primer for A05-216 assay (A05-216R)
gctgccttgccgcttctaa

SEQ ID NO: 3 - DNA, 21 bp, Artificial Sequence
  Forward primer for A02-258 assay (A02-258F)
cattgagcagtgaacaccaag

SEQ ID NO: 4 - DNA, 27 bp, Artificial Sequence
  Reverse primer for A02-258 assay (A02-258R)
cagtttaaactatcagtgtttgaacac

SEQ ID NO: 5 - DNA, 18 bp, Artificial Sequence
  Forward primer for internal reference gene HMG as control (Hmg206F)
tccttccgtttcctcgcc

SEQ ID NO: 6 - DNA, 18 bp, Artificial Sequence
  Reverse primer for internal reference gene HMG as control (Hmg206R)
ttccacgccctctccgct

SEQ ID NO: 7 - DNA, 399 bp, Artificial Sequence
  Transgene junction region of NS-B50027-4 chromosome A05 for assay A05-216
acaagccttgttggcggcggagaagtgatcggcgcggcgagaagcagcggactcggagacgaggccttggaagatctgagtcgaacgggcggtaccgcggccgcaagctttccgcggggcgcccgttttacaacgtcgtgactgggagatccactagcagattgtcgtttcccgccttcagtttaaactatcagtgtttgaaggacagacccacccaagaacacaccagtcattcagatgcagcctatctccgtgccggctattccagctgagagttgaaggatataactgataactatggttccaagtccttgattggtgagggctcttatggaagagtgttttacggtgttcttagaagcggcaaggcagctgccattaagaagctggattctagta

SEQ ID NO: 8 - DNA, 380 bp, Artificial Sequence
  Transgene junction region of NS-B50027-4 chromosome A02 for assay A02-258
tttctttacccaaatctagttcttgagaggatgaagcatcaccgaacagttctgcaactatccctcaaaagctttaaaatgaacaacaaggaacagagcaacgttccaaagatcccaaacgaaacatattatctatactaatactatattattaattactactgcccggaatcacaatccctgaatgattcctattaactacaagccttgttggcggcggagaagtgatcggcgcggcgagaagcagcggactcggagacgaggccttggaagatctgagtcgaacgggcggtaccgcgggcccgttttacaacgtcgtgactgggagatccactagcagattgtcgtttcccgccttcagtttaaactatcagtgtttg

SEQ ID NO: 9 - DNA, 20 bp, Artificial Sequence
  Forward primer for junction between T-DNA and genomic DNA on chromosome A05 (A05-200F)
tgttgtggtggtgacgattt

SEQ ID NO: 10 - DNA, 21 bp, Artificial Sequence
  Reverse primer for junction between T-DNA and genomic DNA on chromosome A05 (A05-200R)
tccactagcagattgtcgttt

SEQ ID NO: 11 - DNA, 640 bp, Artificial Sequence
  Transgene junction region of NS-B50027-4 chromosome A05 for assay A05-200
taatcatggaggagaagaaggatttttataaccatgtctctgttgcttgctgcttaaaccctatataattggaaactttttgttttagtctgtgtctgaaagtttctatattcgtattgtctattttgtaaagactaaaacaaaaatgcctatttttagtttgttcttgttccgcaacaccgttactgaactcttcgttcacttaaacagtttgtgtgtgtgagaaacagcgtaatgagctgctttggttgttgtggtggtgacgattttcgtcgagttgctgaaactggacccaagccagtgtacggcgcaggaggtactttaagcttataaccctttgtctatcctttggctagcggctaatgttgatgaacttttttattcaaccgttggctaaggtaacactgatagtttaaactgaaggcgggaaacgacaatctgctagtggatctcccagtcacgacgttgtaaaacgggcgccccgcggaaagcttgcggccgcggtaccgcccgttcgactcagatcttccaaggcctcgtctccgagtccgctgcttctcgccgcgccgatcacttctccgccgccaacaaggcttgtagttaataggaatcattcagggattgtgattccgggcagtag